European Patent Application EP 4 424 821 A1, published September 4, 2024. Title: Enzymatic synthesis of odilorhabdin and related peptides/proteins comprising non-standard amino acid residues. Applicant: Max-Planck-Gesellschaft zur Förderung der Wissenschaften e.V. Application EP. The sequence listing filed with the application follows.

SEQUENCE LISTING (48 sequences)

SEQ ID NO: 1 - protein, 285 aa, Xenorhabdus nematophila
  source 1..285: note = protein encoded by odlB gene from Xenorhabdus nematophila
MGCVVEVTRFDQNECHRTLAQGCAIVFRGLLKDWPAIERWGADYFQAKCPQIDVIIKFFDADGVRFEPAKMYRYLELLNEYKKGEKGGSIPYCHDIPIFLQAQQLLDDIGDFPLMALPKLYREDWWQFVQFFMSPAGAVTPLHFDTLRTNNLFFQIQGSKRFTFIPWEERNACSRRGWRWFEYNPEIQGDNKFVNISNCTIEVHQGDMLLMPAGMLHHVRTLTDSISFNIDFHTRSSAIASFKSIKEKMPRENLYYNGLSLCGLLGLIKRERFFEKYRPYLNYIS

SEQ ID NO: 2 - protein, 247 aa, Xenorhabdus nematophila
  source 1..247: note = protein encoded by odlE gene from Xenorhabdus nematophila
MLELFEDQLVEIKEKYGHDCLKRVEDMFYPLLQQRSPLQADAKYIMPGLSTTPWLETNDFPQLQPLVTALMKSAGKIKQEMNAVMSGECEYVIDYEHYLGTQKDWKALYLFKNGQPNSAIANILPATWYIFNNELRDWHCPLLEVHFSVLQPGTVIKPHCDLWNFTLNLHFAVDIPASNCQIIVANEARNWQEGECLLFDYSYQHEAYNRSDKHRICLLMDIWHPNLSFAEREALVLIFTGIRKLFG

SEQ ID NO: 3 - protein, 319 aa, Xenorhabdus nematophila
  source 1..319: note = protein encoded by odlF gene from Xenorhabdus nematophila
MMPDTQEVSDFIFELNPTELISLTQMFSESDLKYDIDNFEDFYWKCFQYSFNLPERLQKRLFNFRALENKNYLLIKGLPVPDNLSLTPLSYEQTNSPEVASVRTLISTILSRIGYIYSFVNKKNFNFIDDIFPIEKYKDMQLGTNKKFLEWHVEDGFHDAKADWVALYCLRGDINAETYLFQTKNIHLDAETVSELQKPNFEIDADPTFMSDTDGCRRIAVLSQHKEPEIVFDPAYMRCLTPNSEIALKKLNQCIDENREAFILSPGEMLLFDNRKVAHARSEYEPRYDGYDRWLLRALILESKFKARDHFYAGTLRAK

SEQ ID NO: 4 - protein, 801 aa, Xenorhabdus nematophila
  source 1..801: note = protein encoded by odlG gene from Xenorhabdus nematophila
MIMTSFKTIILLLTILLIIGCGESNSYPIKEAAPTFEARIVRTHYGVPHIYAKSLGSLSFGNAYAQAQDNICIMADNYVRVKGERARFFGPDKEKKGDALNLIQDFGYKSLAFVEQASEKWSQLSPDSQEIIDGFVAGYNTYLSHVKEGRYSLPKACRDQEWVVPVRREDVLAYLFSIAAFPGSERFMADYYAANPNNTGDQKQLASSQHDDHGYSIGSNAWALGHDKIEQGNGMLLANPHFPYEGDMRFWQAHHVVDGKIDVMGASLVGFPGVINIGFNRHIAWTHTYSSAEHVVVYKMQTADNNPLSYVIDGVVRPVKSKPVHIEFKSDNGIQTITKDHFYTDIGPIIENEDFIWSESEFYVVKDINLYNLDMIDHWLALNRANSLAEVKQSYKDFNGLVFNNTLLTGREDVGVFMGDKAVPALSFEAIQLLKNDEMWSAARKEYGVTILPGHLSSMIFTAALGYDQTPQLVKSSYVQNANDSHWATNPKHLLEGFSPLLGNERSPLSFRTRMGLQLIEDAAGDDKKFSLMELEQALLSDRSYLAELILKDVVALCDETPNKLINMMNKVKVDITQACQLLSEWNGEFNADSRGAIVFRELAFLIDQQEHFSVPFDMAYPATTPRQLKQNEEIITLLARAVINVNNVGLDLDTPVNKFQFIESTAPDGKPAGNRMSWPGVFEEEGGFNMIATSDWDKTLFPKHHYPVGNDVVSGEELESQLTDQGYHVRFGSSWSMLVEFNQQGPNARGLLTYSQSSDLDSPHFADQSLFYSRYKQLLPLPYRSEEIKQSTISELIIQH

SEQ ID NO: 5 - protein, 433 aa, Xenorhabdus nematophila
  source 1..433: note = domain of non-ribosomal peptide synthetase from Xenorhabdus nematophila having a L-3-hydroxyarginine dehydratase activity
DVYPLSSLQMGSIYHQLKDESYHIVEHYAINAEWNEQAFYQVFNAIVQRHELLRVAYNFKLGRALQYVRKTVALPIVLNDWRNLSAQEFEHQLGYCLEQENNHFFVEDELMWRVNVLIDAGNTFVLVLSHQHAILDGWSVANLTVEFMGNYLSVSSGGAVPLRADLPHYGEYIAEELAAIDSPEQKTYWQHIANAAVLPDWTGKESTQHYASRLELSYLHDDLQQLAGRLNVPLRTLLLAVHVYVLAKVNGTDSITSSVVSHGRLEVEGAEACLGLFLNTPPVNANIDQQTWASLIQQLTEYNTASWPYRHYPVAMMQEVFKCDYSGALFNYVDFHVADELQATQDAESEQIYEHEHEHEYERVDYGYDLVCHHSSASGFLALQLALTQSVFKAHQVSQILAYYETAIKSMLVSQHHRLAHTDYLAPGQIQHL

SEQ ID NO: 6 - DNA, 25 bp, synthetic construct
  source 1..25: mol_type = other DNA; note = pc1214
ttttgttatcaataaaaaaggcccc

SEQ ID NO: 7 - DNA, 46 bp, synthetic construct
  source 1..46: mol_type = other DNA; note = pc1234
tatacgagccgatgattaattgtcactagtatttcccctctttctc

SEQ ID NO: 8 - DNA, 42 bp, synthetic construct
  source 1..42: mol_type = other DNA; note = pc1216
tgacaattaatcatcggctcgtataatgtgtggaattgtgag

SEQ ID NO: 9 - DNA, 43 bp, synthetic construct
  source 1..43: mol_type = other DNA; note = pc1215
ggggccttttttattgataacaaaattgtctagagcggttcag

SEQ ID NO: 10 - DNA, 45 bp, synthetic construct
  source 1..45: mol_type = other DNA; note = pc1075
tgggctaacaggaggaattccatgtttctagataaagtcgggcag

SEQ ID NO: 11 - DNA, 48 bp, synthetic construct
  source 1..48: mol_type = other DNA; note = pc1105
tgactgccaacagcgagtgaccgccgaggtggaaaaagttgtcgtttc

SEQ ID NO: 12 - DNA, 22 bp, synthetic construct
  source 1..22: mol_type = other DNA; note = pc1106
ggcggtcactcgctgttggcag

SEQ ID NO: 13 - DNA, 24 bp, synthetic construct
  source 1..24: mol_type = other DNA; note = pc1102
gccagtgccaacgaggcatattcg

SEQ ID NO: 14 - DNA, 24 bp, synthetic construct
  source 1..24: mol_type = other DNA; note = pc1103
cgaatatgcctcgttggcactggc

SEQ ID NO: 15 - DNA, 46 bp, synthetic construct
  source 1..46: mol_type = other DNA; note = pc1104
atacgagccgatgattaattgtcacagcgcctccgcttcacaattc

SEQ ID NO: 16 - DNA, 30 bp, synthetic construct
  source 1..30: mol_type = other DNA; note = pc1091
tgacaattaatcatcggctcgtataatgtg

SEQ ID NO: 17 - DNA, 29 bp, synthetic construct
  source 1..29: mol_type = other DNA; note = pc1090
ggaattcctcctgttagcccaaaaaaacg

SEQ ID NO: 18 - DNA, 52 bp, synthetic construct
  source 1..52: mol_type = other DNA; note = pc1080
tttttgggctaacaggaggaattccatgaatatgacacgtaaccatacatcc

SEQ ID NO: 19 - DNA, 31 bp, synthetic construct
  source 1..31: mol_type = other DNA; note = pc1197
cccccaagctcaaagaaatgatcgtggcgac

SEQ ID NO: 20 - DNA, 50 bp, synthetic construct
  source 1..50: mol_type = other DNA; note = pc1198
acgatcatttctttgagcttgggggtcactctttattaattatgtcattg

SEQ ID NO: 21 - DNA, 49 bp, synthetic construct
  source 1..49: mol_type = other DNA; note = pc1246
gtaccgcaagcaacgaatggccccccaaagcaaaaaagttgtcatggcg

SEQ ID NO: 22 - DNA, 25 bp, synthetic construct
  source 1..25: mol_type = other DNA; note = pc1245
gggggccattcgttgcttgcggtac

SEQ ID NO: 23 - DNA, 48 bp, synthetic construct
  source 1..48: mol_type = other DNA; note = pc1247
gtaccgcaagcaacgaatggcccccaagctcaaagaaatgatcgtggc

SEQ ID NO: 24 - DNA, 49 bp, synthetic construct
  source 1..49: mol_type = other DNA; note = pc1242
tttttgggctaacaggaggaattccatgcctatgtcgtgcaatcgtatc

SEQ ID NO: 25 - DNA, 49 bp, synthetic construct
  source 1..49: mol_type = other DNA; note = pc1248
gtaccgcaagcaacgaatggccccccaattcaaagaaatggtcacggcg

SEQ ID NO: 26 - DNA, 22 bp, synthetic construct
  source 1..22: mol_type = other DNA; note = pc1078
gttgtcataccgactgatccgc

SEQ ID NO: 27 - DNA, 42 bp, synthetic construct
  source 1..42: mol_type = other DNA; note = pc1128
tgagcggatcagtcggtatgacaactttttcaggctcggagg

SEQ ID NO: 28 - DNA, 50 bp, synthetic construct
  source 1..50: mol_type = other DNA; note = pc1079
tacgagccgatgattaattgtcactcattattatgcctgctttgtttttc

SEQ ID NO: 29 - DNA, 28 bp, synthetic construct
  source 1..28: mol_type = other DNA; note = pc1210
cgccgacagattacgccaatcattgagc

SEQ ID NO: 30 - DNA, 28 bp, synthetic construct
  source 1..28: mol_type = other DNA; note = pc1211
gctcaatgattggcgtaatctgtcggcg

SEQ ID NO: 31 - DNA, 44 bp, synthetic construct
  source 1..44: mol_type = other DNA; note = pc1231
tatacgagccgatgattaattgtcattgttgccgttgtttgcac

SEQ ID NO: 32 - DNA, 28 bp, synthetic construct
  source 1..28: mol_type = other DNA; note = pc1230
ccacagcatcccccaccagccgataatg

SEQ ID NO: 33 - DNA, 43 bp, synthetic construct
  source 1..43: mol_type = other DNA; note = pc1229
tatcggctggtgggggatgctgtgggggcatgtgttgctttcg

SEQ ID NO: 34 - DNA, 25 bp, synthetic construct
  source 1..25: mol_type = other DNA; note = pc1238
cagaatcccccaccagccgataatg

SEQ ID NO: 35 - DNA, 43 bp, synthetic construct
  source 1..43: mol_type = other DNA; note = pc1239
tatcggctggtgggggattctgtgggggcatgtgttgctttcg

SEQ ID NO: 36 - DNA, 50 bp, synthetic construct
  source 1..50: mol_type = other DNA; note = pc1205
catagcgagcagcgaatgtccacctaaagcgaagaaattatcgtaacgac

SEQ ID NO: 37 - DNA, 25 bp, synthetic construct
  source 1..25: mol_type = other DNA; note = pc1206
ggtggacattcgctgctcgctatgc

SEQ ID NO: 38 - DNA, 50 bp, synthetic construct
  source 1..50: mol_type = other DNA; note = pc1235
gcatagcgagcagcgaatgtccacccatttccataaaagatgcggttaag

SEQ ID NO: 39 - DNA, 46 bp, synthetic construct
  source 1..46: mol_type = other DNA; note = pc1098
tttttgggctaacaggaggaattccatgggctgtgtagtagaagtg

SEQ ID NO: 40 - DNA, 53 bp, synthetic construct
  source 1..53: mol_type = other DNA; note = pc1099
tatacgagccgatgattaattgtcaagaaatataattaaggtacggacggtac

SEQ ID NO: 41 - DNA, 48 bp, synthetic construct
  source 1..48: mol_type = other DNA; note = pc1096
ttttttgggctaacaggaggaattccatgatgcctgatactcaggaag

SEQ ID NO: 42 - DNA, 45 bp, synthetic construct
  source 1..45: mol_type = other DNA; note = pc1097
tatacgagccgatgattaattgtcatttcgcccttaaagtacctg

SEQ ID NO: 43 - DNA, 55 bp, synthetic construct
  source 1..55: mol_type = other DNA; note = pc1088
gtttttttgggctaacaggaggaattccatgttggaactatttgaagatcaattg

SEQ ID NO: 44 - DNA, 48 bp, synthetic construct
  source 1..48: mol_type = other DNA; note = pc1222
tttttgggctaacaggaggaattccatgataatgacatcatttaagac

SEQ ID NO: 45 - DNA, 50 bp, synthetic construct
  source 1..50: mol_type = other DNA; note = pc1223
tatacgagccgatgattaattgtcaatgttgaataattaactctgaaatc

SEQ ID NO: 46 - DNA, 48 bp, synthetic construct
  source 1..48: mol_type = other DNA; note = pc1236
actagagaaagaggggaaatactagatgataatgacatcatttaagac

SEQ ID NO: 47 - DNA, 21 bp, synthetic construct
  source 1..21: mol_type = other DNA; note = pc1213
ctagtatttcccctctttctc

SEQ ID NO: 48 - DNA, 1095 bp, synthetic construct
  source 1..1095: mol_type = other DNA; note = Vaniline promoter sequence
ttttgttatcaataaaaaaggccccccgatttgggaggcctttttagttagaggatccttatcaatctgcacgaattgaccatgctgcacccagcggtgcgcctgcgcttgctgctgcttcaaaaacttttgcattacgaattgctgccagtgcatgatcacgcataatacgttctgcaccttcggcatcaccacagctaactgcatccagaactgcctgatgctgacgatgtgctgccagcagatgttcatattcggcagacaggtccatcagatccagggccagtgcaccggctgctgcaaacggttcaaaaccattacgtgccagtgcgctttcaactgcaccattacctgctgcgctaaccagggtatcatgaaatgcctgattatatgcggcataacgatccagatcttcaccattcaggcgaccggctgcaaacagtgcttcaccttctgcaatcagtacaacaaaacgtgcatgggtttctgcggtcataccacgttctgccagacgacgtgctgcaaaaccttccagaacaccacgaacttcaattgcatcacgaatctgatcgctgctaacaccacgggctgcataaccacgtgcacccagacgaacaaccagaccttcttgttccagtgaacgcagtgcgatacgaaccggcatacggctaacacccagtgctgctgcggtcggaatttctgcaatacgttcaccacttttgatttcaccgcttgcaatcattttacgcagtgccatcataacacgctgacccggtttaatacgaggcatgtccattattcacccccctgaattgactctcttccgctagcactgtacctaggactgagctagccgtcaacattggaccaaaacgaaaaaaggcccccctttcgggaggcctcttttctggaatttggtaccgaggcttaacgatcgttggctgattggatccaattgacagctagctcagtcctaggtaccattggatccaatagctgtcaccggatgtgctttccggtctgatgagtccgtgaggacgaaacagcctctacaaataattttgtttaatactagagaaagaggggaaatactag